European Patent Specification EP 3 464 537 B1, published December 11, 2024. Title: Cleaning Compositions comprising Enzymes. Applicant: Novozymes A/S. The sequence listing filed with the application follows.

SEQUENCE LISTING (20 sequences)

SEQ ID NO: 1 - DNA, 732 bp, Aspergillus oryzae
atgcagcttactaagtccctcctggtattcgcgctttacatgtttggcactcagcacgttctagctgtgcctgtcaatcccgagcctgatgctacgagcgtcgaaaatgttgcccttaaaacaggcagcggtgatagccagagcgatcccatcaaggcggacttggaggtcaaaggccaaagtgctttgcctttcgacgtcgactgctgggctatcctgtgcaagggcgccccgaatgtcctgcagcgcgtgaatgaaaagacgaaaaatagtaatcgcgatcggagcggtgcgaacaaagggcctttcaaagatcctcagaaatggggcatcaaagcccttccacctaagaatccatcctggagcgcacaagacttcaaatcacccgaagaatacgcatttgcgtcttcccttcaaggcggaaccaatgccatcctagcgcccgtcaacctcgcttctcagaactcccaaggcggcgtcttgaacggtttctactcggcgaacaaagtagcacaatttgatcctagcaagccccaacagacaaagggaacatggtttcagatcactaagttcacaggtgcagctggtccttactgcaaggctctggggagtaatgataagagtgtgtgcgataagaacaagaatattgcaggggactggggcttcgacccggcgaaatgggcatatcagtatgatgagaagaataacaagttcaactatgttggtaagtaa

SEQ ID NO: 2 - protein, 221 aa, Aspergillus oryzae
VPVNPEPDATSVENVALKTGSGDSQSDPIKADLEVKGQSALPFDVDCWAILCKGAPNVLQRVNEKTKNSNRDRSGANKGPFKDPQKWGIKALPPKNPSWSAQDFKSPEEYAFASSLQGGTNAILAPVNLASQNSQGGVLNGFYSANKVAQFDPSKPQQTKGTWFQITKFTGAAGPYCKALGSNDKSVCDKNKNIAGDWGFDPAKWAYQYDEKNNKFNYVGK

SEQ ID NO: 3 - protein, 351 aa, Actinobacillus pleuropneumoniae
MDLPKKESGLTLDIARRFYTVDTIKQFIDTIHQAGGTFLHLHFSDHENYALESSYLEQREENATEKNGTYFNPKTNKPFLTYKQLNEIIYYAKERNIEIVPEVDSPNHMTAIFDLLTLKHGKEYVKGLKSPYIAEEIDINNPEAVEVIKTLIGEVIYIFGHSSRHFHIGGDEFSYAVENNHEFIRYVNTLNDFINSKGLITRVWNDGLIKNNLSELNKNIEITYWSYDGDAQAKEDIQYRREIRADLPELLANGFKVLNYNSYYLYFVPKSGSNIHNDGKYAAEDVLNNWTLGKWDGKNSSNHVQNTQNIIGSSLSIWGERSSALNEQTIQQASKNLLKAVIQKTNDPKSH

SEQ ID NO: 4 - protein, 359 aa, Aggregatibacter actinomycetemcomitans
CVKGNSIHPQKTSTKQTGLMLDIARHFYSPEVIKSFIDTISLSGGNFLHLHFSDHENYAIESHLLNQRAENAVQGKDGIYINPYTGKPFLSYRQLDDIKAYAKAKGIELIPELDSPNHMTAIFKLVQKDRGIKYLQGLKSRQVDDEIDITNADSIAFMQSLMSEVIDIFGDTSQHFHIGGDEFGYSVESNHEFITYANKLSYFLEKKGLKTRMWNDGLIKSTFEQINPNIEITYWSYDGDTQDKNEAAERRDMRVSLPELLAKGFTVLNYNSYYLYIVPKASPTFSQDAAFAAKDVIKNWDLGVWDGRNTKNRVQNTHEIAGAALSIWGEDAKALKDETIQKNTKSLLEAVIHKANGDE

SEQ ID NO: 5 - protein, 346 aa, Haemophilus sputorum
QNSTKQSGLMLDISRRFYSVETIKQFIDDIAQANGTFLHLHFADHENYALESTFLNQRAENAIVQNGIYINPKTNKPFLTYEQIDQIIRYAQEKQIELIPEVDSPAHIKGILTLLRLEKGEDYVNQIALNQDELNLDSPESLTMMKTLVDEVCYIFGYSAQHFHIGGDEFNYASNFIRYVNALNQHINQKGLITRMWNDGLLQQNIDELDKNIEITYWSFDGDAQEKNDIVERRATRISLPTLLDKGFKALNYNSYYLYFIPKDNGNIATDAKFALNDLKQNWQLLRWDGNYETQPIQQAENLIGAAFSIWGEHAGKLSDDVIHQATSPLIQATIIQTNAKTTGPN

SEQ ID NO: 6 - protein, 352 aa, Actinobacillus suis
MNHSQIKEAGLTLDIARRFYPVETIKQFIDTIHHAGGTFLHLHFSDHENYALESTYLDQSEANAIVKDGTYYNPKTNKPFLTYKQIHDIIYYAKSKNIELVPEVDTPNHMTAIFRLLEAKHGKDYVKKLKSKMNDEEIDITNPESIEVIKTLIAEVIYIFGHASEHFHIGGDEFGYSVETNHEFISYVNTLNQFINEKGKITRIWNDGLIKNNLNQLNKNVEITYWSYDGDAQESQDIAERRKIRANLPELLENGFKVLNYNSYYLYFVPKGNANITHDSKYATEDVLNNWKLGLWDGQNKENMVENTKNIIGSSLSIWGERSGSLSSEVIEESTQDLLKAVIQKTNDPKSH

SEQ ID NO: 7 - protein, 352 aa, Actinobacillus capsulatus
MNHSQIKEAGLTLDIARRFYPVETIKQFIDTIHHAGGTFLHLHFSDHENYALESTYLDQLEANAIVKDGTYYNPTTNKPFLTYKQINDIIYYAKSKNIELVPEVDTPNHMTAIFRLLEAKHSKDYVKRLKSKMNDEEIDITNLESIEVIKTLIAEVIYIFGHASEHFHIGGDEFGYSVETNHEFITYVNTLNQFINNKGKITRIWNDGLIKNNLNQLNKNVEITYWSYDGDAQESQDIAERRKIRVNLPELLENGFKVLNYNSYYLYFVPKGNANITHDSKHATEDVLKNWKLGLWDGQNKENIVENTKNIIGSSLSIWGEHSGSLSSAVIEESTQELLKAVIQKTNDPKSH

SEQ ID NO: 8 - protein, 352 aa, Actinobacillus equuli subsp. equuli
MNHSQIKEAGLTLDIARRFYPVETIKQFIDTIHHAGGTFLHLHFSDHENYALESSYLDQSEENAIVKDGTYYNPKTNKPFLTYKQIDDIIYYAKSKNIELVPEVDTPNHMTAIFNLLEIKHGEAYVKNLKSKMNDEEIDITNPESIEVIKTLIAEVIYIFGHASEHFHIGGDEFGYSVETNHEFISYVNTLNQFINEKGKITRIWNDGLIKNNLNQLNKNVEITYWSYDGDAQKSQDIAERRKIRADLPELLENGFKVLNYNSYYLYFVPKGNANITHDSKYATEDVLNNWKLGLWDGKNKENEVKNTKNIIGSSLSIWGERSGSLSSEVIEESTQDLLKAVIQKTNDPKSH

SEQ ID NO: 9 - protein, 359 aa, Aggregatibacter actinomycetemcomitans
CVKGNSIYPQKISTKQTGLMLDIARHFYSPEVIKSFIDTISLSGGNFLHLHFSDHENYAIESHLLNQRAENAVQGKDGIYINPYTGKPFLSYRQLDDIKAYAKAKGIELIPELDSPNHMTAIFKLVQKDRGVKYLQGLKSRQVDDEIDITNADSIAFMQSLMNEVIDIFGDTSQHFHIGGDEFGYSVESNHEFITYANKLSYFLEKKGLKTRMWNDGLIKSTFEQINPNIEITYWSYDGDTQDKNEAAERRDMRVSLPELLAKGFTVLNYNSYYLYIVPKASPTFSQDAAFAAKDVIKNWDLGVWDGRNTKNRVQNTHEIAGAALSIWGEDAKALKDETIQKNTKSLLEAVIHKTNGDE

SEQ ID NO: 10 - protein, 359 aa, Aggregatibacter actinomycetemcomitans
CVKGNSIYPQKTSTKQTGLMLDIARHFYSPEVIKSFIDTISLSGGNFLHLHFSDHENYAIESHLLNQRAENAVQGKDGIYINPYTGKPFLSYRQLDDIKAYAKAKGIELIPELDSPNHMTAIFKLVQKDRGVKYLQGLKSRQVDDEIDITNADSITFMQSLMSEVIDIFGDTSQHFHIGGDEFGYSVESNHEFITYANKLSYFLEKKGLKTRMWNDGLIKNTFEQINPNIEITYWSYDGDTQDKNEAAERRDMRVSLPELLAKGFTVLNYNSYYLYIVPKASPTFSQDAAFAAKDVIKNWDLGVWDGRNTKNRVQNTHEIAGAALSIWGEDAKALKDETIQKNTKSLLEAVIHKTNGDE

SEQ ID NO: 11 - protein, 461 aa, Curtobacterium oceanosedimentum
ADRNTSAAEAAVTSIAPRATITGVAAISAATSSRTTVRTTLTLENRSGERESAADAWLYLAGGGARYALGHAPVRALAAGARATVRTTLRVPSRAPAGKYAVLACAGPYSKQACRTSGTTVTVGTAARARPETGVMLDVARAYYPVSLIEQYVDLLAEHGGGFLHLHLTDDQNVGIESAVLGQTPANAVLRNGVYTSRVTGRPFLSAAQARAISAYAAKRGIAIVPEVDSPGHMAAAFALLEARHGATWVDRIRSGESELDTSVPESATLAAELLREVTQTFPSSRTVHIGGDEWGADVSADERVGWMNAMAAAIGDREVWAWNDGIDRASVGRLDPRIHVTYWSFDGDTEDAAERRERRARRASATDLQRAGIDLLNYNSYYLYEVPTDLDPADSEYTVADLREHWSLRAWDGDSGARLAAPMSGAAVAIWGEDLDGAPSEALLRWSAPHVTAMIETAAS

SEQ ID NO: 12 - protein, 324 aa, Terribacillus saccharophilus
QDQEKGITIDISRKYYSIKTLKAIVDEISANGGDYLQLHFSDNESYAIASEFLGQNSENPNSAYLTKKELLSLIAYSNDRNIMVIPDIDLPAHSKGWLNIMKEKDSGLYTDIVTDYSEDTLDYHNNAVALYTANQLLDEVLDLFYQPKFAGKQRIVLGGDEVPGSGAHQTDFIRFMNQIAKTAKASNYEPQMWNDSITPEGIQNLDRSFSILYWKQSTLSNGAQSLDVQDFEENGLSVYNYNAYSLYFLPSTRFTQEDITEQIDYMKWAYAYNKFFYISDYYKQVDTPNVKGSSLVFWGEHANDLSQEGLLKQEKPLIQNFLGL

SEQ ID NO: 13 - protein, 324 aa, Terribacillus goriensis
QDQEKGITIDISRKYYSIETLKSIIDEISANGGDYLQLHFSDNERYAIASEFLGQNGENPNSTYLTKKELLSLIAYSNDRDIMVIPDIDLPAHSRGWLNIMKEKDSGLYTDIVTDYSEDTLDYHNNAVALYTANQLLDEVLDLFYQPKFAGKQRIVLGGDEVPGSGVHQTDFIRFMNQIAETAKASNYKPQMWNDSITPEGIQNLDRSFSILYWKQSTLSNGAQGLDVQDFEENGLSVYNYNAYSLYFLPATRFTQEDITEQIDYMKWAYAYNKFFYISDYYKQVDTSNVKGSSLVFWGEHANDLSQEGLLKQEKPLIQNFLGL

SEQ ID NO: 14 - protein, 324 aa, Terribacillus saccharophilus
KDQEKGITIDISRKYYSIGTLKAIVDEINANGGDYLQLHFSDNESYAIASEFLGQNSENPNSTYLTKKELLSLIAYSNDRNIMVIPDIDLPAHSKGWLNVMKEKDSGLYTDIVTDYSEDTLDYHNNAAALYTANQLLDEVLDLFYQPKFAGKQRIVLGGDEVPGSGAHQTDFIRFMNQIDETAKASNYEPQMWNDSITPEGIQNLDRSFSILYWKQSTLSSGAQGLDVQNFEEKGFSVYNYNAYSLYFLPSTRFTQEDITEQIDYMKWAYAYNKFFYISDYYKQVDTSNVKGSSLVFWGEHANDLSQEGLLEQEKPLIQNFLSL

SEQ ID NO: 15 - protein, 445 aa, Curtobacterium flaccumfaciens
DTAVSAVTVTKVTASTTGTVVRTTLKVENTAPVRKPASSVWLYLSAGTEKYTLGRVAVKALAAGSSTSVTAVRGTPSRAAAGKYSVLACAGAYSAKQCRTSTATVTTKPTKRARPETGVMLDVARAYYPVALIKRYIDLLADDGGRFLHLHLTDDQNVGIESTVLGQTPANADLDHGVYTSRVTHRPFLSAAQARTISAYGAERGVAIVPEIDTPGHMAAAFALLEAQHGTKWVDRIRSGENELDTSAPESLALAKKLYAEVQRTFPSSRTVHIGGDEWGDDVTAAQRVTWMNAMAAALDDREVWAWNDGIDRVAVGRLDPRIHVTYWSFDGDTEDAAERRERRARRASAVDLQQAGIDQLNYNSYYLYEVPTDLDPADSDYTVADLRENWSLRAWDGDSGSLLAAPMSGAAVAIWGEDLEDPPSDALLRWSAPHVTAMIETAAS

SEQ ID NO: 16 - protein, 445 aa, Curtobacterium luteum
DTAVSAVTVTKVTASTTGTAVRTTLKVENTAPVRKPASSVWLYLSAGTEKYTLGRVAVKALSAGSSTSVTAVRGTPSRAAAGKYWVLACAGAYSAKQCRTSTATVTTKPTKRARPETGVMLDVARAYYPVALIKRYIDLLADDGGRFLHLHLTDDQNVGIESTVLGQTPANADLDHGVYTSRVTHRPFLSAAQARTISEYGAERGVTIVPEIDTPGHMAAAFALLEAQHGTKWVDRIRSGENELDTSAPESLVLAKKLYAEVQRTFPSSRTVHIGGDEWGDDVTAAHRVAWMNEMAATLGNREVWAWNDGIDRVAVGRLDPRIHVTYWSFDGDTEDAAERRERRARRASAVDLQQAGIDQLNYNSYYLYEVPTDLDPADSDYTVADLRENWSLRAWDGDSGSLLAAPMSGAAVAIWGEDLEDPPSDALLRWSAPHVTAMIETAAS

SEQ ID NO: 17 - protein, 458 aa, Curtobacterium oceanosedimentum
IGGSAGTADASGAPRLVVTKVTASSTTTSTRTTVRTTLTVKNTSVARKPAADAWLSLTAGSKRYTLGHVSVQSLAAGASATIHATHTAPPRAPAGKYAVLACTGAFSLSKCGTSATTVTTARATRARPDTGVMLDVARAYYPVALIEQYIALLADHGGRFLHLHLTDDQNVGIESEVLGQTLANADLRDGVYTSRITGRPFLSAAQAREISRYAAQRGIAIIPEIDTPGHMAAAFALLEAGHGKQWVDRIRSGESELDTSAPGSSALAARLLQEVTRTFPSSRTVHIGGDEWGDDVTADERVQWLNTMAAAVGNRAVWAWNDGIDRAAIGRLDPRIHVTYWSFDGDTEDATERRERRERRAGANDLYAAGIDLLNYNSYYLYEVPTDLDAADSEYTVADLRENWSLRTWDGDSGARLAGPTSGAAVAIWGEDLEAPPSDALLRWSAPHVLAMIETAGS

SEQ ID NO: 18 - protein, 450 aa, Curtobacterium sp. Leaf154
AGSTTSTVTVTQVTATTTASSTGTAVRTTLKIKNTAAVRKPASSAWLYLSAGTKKYTLGRVAVKALAAGSSTSVTAVRGTPSRATAGEYSVLACAGAYSAKQCRTSTATVTTKPTKRARPETGVMLDVARAYYPVALIKRYIDLLADDGGRFLHLHLTDDQNVGIESTVLGQTLANADLDEGVYTSRVTRRPFLSAAQARTISDYAARRGVAIVPEIDTPGHMTAAFDLLEAQHGTKWVDRIRSGENELDTSTPGSLALAKKLYAEVQRTFPASRTVHIGGDEWGDDVSAAERVAWMNAMAAALGNREVWAWNDGIDRVAVGRLDPRIHVTYWSFDGDTEDAAERRERRARRASAVDLQQAGIDMLNYNSYYLYEVPTDLDPADSEYTVADLRENWSLRTWDGDSGSLLAAPMSGAAVAIWGEDLEDPPSDALLRWSAPHVTAMIETAAS

SEQ ID NO: 19 - protein, 324 aa, Terribacillus saccharophilus [sequence omitted]

SEQ ID NO: 20 - protein, 324 aa, Terribacillus saccharophilus
KDQEKGISIDISRKYYSIGTLKAIIDEISANGGDYLQLHFSDNESYAIASDYLGQISDTPNNTYLTKNDLLSLIAYSNDRNILIIPDMDLPAHSRGWLELMKVKDRELYTDIVTDYSNETLDYHNNTDALNTANQLLNEILELFYQPKFAGKQRIVLGGDEVPGSEIHQLDFIRFINQIASTAKASNYAPQMWNDSITAEGIQNLDKSFSILYWKQSTLSNGAQSLEVQDFEDWDFPVYNYNAYSLYFLPSIRFTDEDITEQMNYMKWAYAYNKFFYISDYYKSVDASNVKGSSLTFWGEHATDLSQEELLEQELPLIKKFLSL